European Patent Application EP 4 335 453 A1, published March 13, 2024. Title: Medical Use of Hypoxia-inducible Lipid Droplet-associated Protein or Truncated Fragment thereof. Applicant: Westlake University. The sequence listing filed with the application follows.

SEQUENCE LISTING (31 sequences)

SEQ ID NO: 1 - protein, 63 aa, Homo sapiens
MKHVLNLYLLGVVLTLLSIFVRVMESLEGLLESPSPGTSWTTRSQLANTEPTKGLPDHPSRSM

SEQ ID NO: 2 - protein, 64 aa, Mus musculus
MKFMLNLYVLGIMLTLLSIFVRVMESLGGLLESPLPGSSWITRGQLANTQPPKGLPDHPSRGVQ

SEQ ID NO: 3 - protein, 63 aa, Chlorocebus sabaeus
MKHMLNLYLLGVVLTLLSIFVRVMESLEGLLENPSPGTSWTTRSQLANTEPTKGLPDHPSRSI

SEQ ID NO: 4 - protein, 63 aa, Rhinopithecus roxellana
MKHVLNLYLLGVVLTLLSIFVRVMESLEGLLENPLPGTSWTTRSQLTNTEPTKGLPDHPSRSM

SEQ ID NO: 5 - protein, 63 aa, Macaca fascicularis
MKHMLNLYLLGVVLTLLSIFVRVMESLEGLLENPSPGTSWTTRSQLANTEPTKGLPDHPSRSM

SEQ ID NO: 6 - protein, 62 aa, Sus scrofa
MKQVLQLYLLGVVLTLLSVFVRLMETLGGLLESPSPGSFWTTRGQLANTEAKSLPEHPSRGV

SEQ ID NO: 7 - protein, 71 aa, Canis familiaris
MKPMLNLYLLGVVLTLLSIFVRLMESLGGILESPLLGSSWTTRGHTASAEPPRAFQTIHPERCDKTSLHQL

SEQ ID NO: 8 - protein, 71 aa, Capra hircus
MKHVLNLYLLGGVLTLLSIFVRLMESLEGLLESPSPGSSWATRGQLANTEPPRAFQTIHPEGCDKTSLHRL

SEQ ID NO: 9 - protein, 71 aa, Equus caballus
MKHILNLYLLGVVLTLLSIFVRLMESLEGLLESPSPGSSWTTRSQLVSTRPPRAFQTIHPEGCDKTSVHRL

SEQ ID NO: 10 - protein, 98 aa, Bos taurus
MKHMLNLYLLGGVMTLLSIFIGLMESLEACWRACLLGAPGPPEVSLPTQSPQGSSRPSIQRGVIRPPSTVYNLGTVSKIPPTLPVPGQASSTSVLSEN

SEQ ID NO: 11 - protein, 64 aa, Oryctolagus cuniculus
MKHVLNLYVLGVVLALLSIFVRVMESLESLVESPSAGNSWSTRGQLAGAEPPKGLPDPPSRGMR

SEQ ID NO: 12 - protein, 64 aa, Rattus norvegicus
MKYMLNLYVLGVMLTLLSIFVRLMESLGGLLENPLPGSSWITRGHLANTQPPRGLPDHPSRGVQ

SEQ ID NO: 13 - protein, 20 aa, Artificial Sequence
  truncated fragment of human HILPDA
MKHVLNLYLLGVVLTLLSIF

SEQ ID NO: 14 - protein, 20 aa, Artificial Sequence
  truncated fragment of rat HILPDA
MKYMLNLYVLGVMLTLLSIF

SEQ ID NO: 15 - protein, 20 aa, Artificial Sequence
  truncated fragment of mouse HILPDA
MKFMLNLYVLGIMLTLLSIF

SEQ ID NO: 16 - DNA, 39 bp, Artificial Sequence
  primer
atagaagattctagaatgaagcatgtgttgaacctctac

SEQ ID NO: 17 - DNA, 42 bp, Artificial Sequence
  primer
cgcggccgcggatcctcacttatcgtcgtcatccttgtaatc

SEQ ID NO: 18 - DNA, 720 bp, Artificial Sequence
  vector pCDH-CMV-MCS-EF1-GFP+Puro
atggtgagcaagggcgaggagctgttcaccggggtggtgcccatcctggtcgagctggacggcgacgtaaacggccacaagttcagcgtgtccggcgagggcgagggcgatgccacctacggcaagctgaccctgaagttcatctgcaccaccggcaagctgcccgtgccctggcccaccctcgtgaccaccctgacctacggcgtgcagtgcttcagccgctaccccgaccacatgaagcagcacgacttcttcaagtccgccatgcccgaaggctacgtccaggagcgcaccatcttcttcaaggacgacggcaactacaagacccgcgccgaggtgaagttcgagggcgacaccctggtgaaccgcatcgagctgaagggcatcgacttcaaggaggacggcaacatcctggggcacaagctggagtacaactacaacagccacaacgtctatatcatggccgacaagcagaagaacggcatcaaggtgaacttcaagatccgccacaacatcgaggacggcagcgtgcagctcgccgaccactaccagcagaacacccccatcggcgacggccccgtgctgctgcccgacaaccactacctgagcacccagtccgccctgagcaaagaccccaacgagaagcgcgatcacatggtcctgctggagttcgtgaccgccgccgggatcactctcggcatggacgagctgtacaagtaa

SEQ ID NO: 19 - DNA, 35 bp, Artificial Sequence
  primer
atagaagattctagaatggtgagcaagggcgagga

SEQ ID NO: 20 - DNA, 62 bp, Artificial Sequence
  primer
cgcggccgcggatccttacttatcgtcgtcatccttgtaatccttgtacagctcgtccatgc

SEQ ID NO: 21 - DNA, 954 bp, Artificial Sequence
  vector pDONR223-APOE
atgaaggttctgtgggctgcgttgctggtcacattcctggcaggatgccaggccaaggtggagcaagcggtggagacagagccggagcccgagctgcgccagcagaccgagtggcagagcggccagcgctgggaactggcactgggtcgcttttgggattacctgcgctgggtgcagacactgtctgagcaggtgcaggaggagctgctcagctcccaggtcacccaggaactgagggcgctgatggacgagaccatgaaggagttgaaggcctacaaatcggaactggaggaacaactgaccccggtggcggaggagacgcgggcacggctgtccaaggagctgcaggcggcgcaggcccggctgggcgcggacatggaggacgtgtgcggccgcctggtgcagtaccgcggcgaggtgcaggccatgctcggccagagcaccgaggagctgcgggtgcgcctcgcctcccacctgcgcaagctgcgtaagcggctcctccgcgatgccgatgacctgcagaagcgcctggcagtgtaccaggccggggcccgcgagggcgccgagcgcggcctcagcgccatccgcgagcgcctggggcccctggtggaacagggccgcgtgcgggccgccactgtgggctccctggccggccagccgctacaggagcgggcccaggcctggggcgagcggctgcgcgcgcggatggaggagatgggcagccggacccgcgaccgcctggacgaggtgaaggagcaggtggcggaggtgcgcgccaagctggaggagcaggcccagcagatacgcctgcaggccgaggccttccaggcccgcctcaagagctggttcgagcccctggtggaagacatgcagcgccagtgggccgggctggtggagaaggtgcaggctgccgtgggcaccagcgccgcccctgtgcccagcgacaatcactga

SEQ ID NO: 22 - DNA, 36 bp, Artificial Sequence
  primer
atagaagattctagaatgaaggttctgtgggctgcg

SEQ ID NO: 23 - DNA, 35 bp, Artificial Sequence
  primer
cttccatggctcgaggtgattgtcgctgggcacag

SEQ ID NO: 24 - DNA, 40 bp, Artificial Sequence
  primer
atgccgatgacctgcagaagtgcctggcagtgtaccaggc

SEQ ID NO: 25 - DNA, 40 bp, Artificial Sequence
  primer
gcctggtacactgccaggcacttctgcaggtcatcggcat

SEQ ID NO: 26 - DNA, 40 bp, Artificial Sequence
  primer
gcgcggacatggaggacgtgcgcggccgcctggtgcagta

SEQ ID NO: 27 - DNA, 40 bp, Artificial Sequence
  primer
tactgcaccaggcggccgcgcacgtcctccatgtccgcgc

SEQ ID NO: 28 - DNA, 954 bp, Artificial Sequence
  APOE2
atgaaggttctgtgggctgcgttgctggtcacattcctggcaggatgccaggccaaggtggagcaagcggtggagacagagccggagcccgagctgcgccagcagaccgagtggcagagcggccagcgctgggaactggcactgggtcgcttttgggattacctgcgctgggtgcagacactgtctgagcaggtgcaggaggagctgctcagctcccaggtcacccaggaactgagggcgctgatggacgagaccatgaaggagttgaaggcctacaaatcggaactggaggaacaactgaccccggtggcggaggagacgcgggcacggctgtccaaggagctgcaggcggcgcaggcccggctgggcgcggacatggaggacgtgtgcggccgcctggtgcagtaccgcggcgaggtgcaggccatgctcggccagagcaccgaggagctgcgggtgcgcctcgcctcccacctgcgcaagctgcgtaagcggctcctccgcgatgccgatgacctgcagaagtgcctggcagtgtaccaggccggggcccgcgagggcgccgagcgcggcctcagcgccatccgcgagcgcctggggcccctggtggaacagggccgcgtgcgggccgccactgtgggctccctggccggccagccgctacaggagcgggcccaggcctggggcgagcggctgcgcgcgcggatggaggagatgggcagccggacccgcgaccgcctggacgaggtgaaggagcaggtggcggaggtgcgcgccaagctggaggagcaggcccagcagatacgcctgcaggccgaggccttccaggcccgcctcaagagctggttcgagcccctggtggaagacatgcagcgccagtgggccgggctggtggagaaggtgcaggctgccgtgggcaccagcgccgcccctgtgcccagcgacaatcactga

SEQ ID NO: 29 - DNA, 954 bp, Artificial Sequence
  APOE4
atgaaggttctgtgggctgcgttgctggtcacattcctggcaggatgccaggccaaggtggagcaagcggtggagacagagccggagcccgagctgcgccagcagaccgagtggcagagcggccagcgctgggaactggcactgggtcgcttttgggattacctgcgctgggtgcagacactgtctgagcaggtgcaggaggagctgctcagctcccaggtcacccaggaactgagggcgctgatggacgagaccatgaaggagttgaaggcctacaaatcggaactggaggaacaactgaccccggtggcggaggagacgcgggcacggctgtccaaggagctgcaggcggcgcaggcccggctgggcgcggacatggaggacgtgcgcggccgcctggtgcagtaccgcggcgaggtgcaggccatgctcggccagagcaccgaggagctgcgggtgcgcctcgcctcccacctgcgcaagctgcgtaagcggctcctccgcgatgccgatgacctgcagaagcgcctggcagtgtaccaggccggggcccgcgagggcgccgagcgcggcctcagcgccatccgcgagcgcctggggcccctggtggaacagggccgcgtgcgggccgccactgtgggctccctggccggccagccgctacaggagcgggcccaggcctggggcgagcggctgcgcgcgcggatggaggagatgggcagccggacccgcgaccgcctggacgaggtgaaggagcaggtggcggaggtgcgcgccaagctggaggagcaggcccagcagatacgcctgcaggccgaggccttccaggcccgcctcaagagctggttcgagcccctggtggaagacatgcagcgccagtgggccgggctggtggagaaggtgcaggctgccgtgggcaccagcgccgcccctgtgcccagcgacaatcactga

SEQ ID NO: 30 - DNA, 93 bp, Artificial Sequence
  3xHA
tacccttatgacgtacctgactatgctggcgcctacccttatgacgtacctgactatgctggatacccttatgacgtacctgactatgcttaa

SEQ ID NO: 31 - DNA, 216 bp, Artificial Sequence
  HILPDA-Flag
atgaagcatgtgttgaacctctacctgttaggtgtggtactgaccctactctccatcttcgttagagtgatggagtccctagagggcttactagagagcccatcgcctgggacctcctggaccaccagaagccaactagccaacacagagcccaccaagggccttccagaccatccatccagaagcatggattacaaggatgacgacgataagtga